European Patent Application EP 4 692 309 A1, published February 11, 2026. Title: 新規ビフィドバクテリウム属細菌. Applicant: 株式会社ヤクルト本社. The sequence listing filed with the application follows.

SEQUENCE LISTING (15 sequences)

SEQ ID NO: 1 - DNA, 2592 bp, Bifidobacterium pseudocatenulatum
  source 1..2592: mol_type = genomic DNA
gtgaaggaggtgcgagcgaacgggttcgggggcagagtagctgccgaaccgaacggcccgatacgcgggctacgcaaggaatacaccattatcaatgaggaaagtgatggatacacattgttcaatacaaccgatgaacgtggggcgtccaagcgccgtggcatcgtcgcggcgcttgcggccgtagccatgctggtgccgctggcattcgctccgtcggctaccgccgcggaaggcgactactccggtggcatcaagggcgagtacaacgctctgggcatcgccgccggtgtggcgaccgaagcctatagcggtctcaatagccaggaacggcaggatacggtgcttgccaacttcaaccagatcactccggaaaactcgatgaagccggaaggctggtacgacggcaatcatgagttcgccatgtccgataacacccggagcctgttgaagttcgccagcgacaacaacatccggatctacggccacgttctggtgtggcactcccagacgcccgactggttcttccaagcggacgaatggtgtgaggacgccaataacaccgccggtgtcaccagctgcccgctggccgacaaggccacgatgcaggagcgtcagcgtcagcacatcgagaacgtcgccaaggcgatctccgatgagttcggtccgttcggcagcgacacgaatcccgtcgtggcgttcgatgtcgtcaacgaaaccgtgaacgacaccgacaatccggacaccaacggcatgcgcaattcgctgtggtaccagacctacgacggtgaggactacatctatgacgcgttcgagaatgcgaacacgtacttcaacgaggtgtacgccgatccttcggacgatcatccggtgacgttgttcatcaacgattacaacaccgagcagtcgggtaagcgcacccggtatgctgccctgctggaccgtatggttgccgaaggcgtgccgttcgacggcatcggccaccagttccatgtgacgttgaccacggcgacctcgaacctggaggccgcgctgaccgacatggaacgcttcaacaagaagcaggccatcaccgaactggacgtgacgaccggaaccccggtcacggaggccaagctcatcgaacagggccagtactactatgaagtaaatcagatcatccaccgtcacgctgcgcagctgttctccgttacggtgtggggcttgatcgacggactgtcctggcgtagtggcgaaggcgctccgctgctgttcgacgacaacctggagaagaagccggcgtacatcggctacatcggtgatagcgccaaccttcccgagccgttgaagagcatgaacgcattcaaggatgacgccgtgggcatcgactcggcgcttcccggtaccgtggccgagtccggcgcgtcctctccgtgggaacgtctttcgctggtcgagatgaccccgtctgcgaatggcgccgtttccggctcgttcaatgtctattggaaggacggctctctggtcgtctacgcggatgtcgccgatgtcagcgcggcggatgacgacaccgtcaccgtgcgtgtgggtgacgccgagtatacgatcggccgcaacggtgtgaccggcggcgagggtgtgcaggccaacgtcgtttcgtctgatgccggatacgaagtcgtggccgatatcccatacaccggtgcagagaaggacatcgtcgagatgaacgtcatcgcgacggattccgccaccacggagaccagcgcgtggagcacgaacgacaccggcgccgtcacgctggccgagccgctgagctacacggaagccgtgaaggttcccgccgacgcccaagctccggtcgttgacgccgacccgtcggatcccgtctgggcggaagccaacgaggttcccgtggataaggtgaccgccgccacgccttcccccgaggcgaccgctaccgccaagaccctgtggtcggacggcaagctgtatgtcctcatggaagtgaccgacgcggacatcgacctgaccaactcgaatccgtgggagaaggactccgtggaggtatacatcgaccgcggcaacaccaagagcggccagtacaccaacgacatccagcagattcgcgtgtccgccgatggcgcggagctgagcttcggctccggcgcgtcggaggatgtccagaagtccatggtccagaccgccggcacgatcgtcgatggcggctatgtcgtcgagatggccatcgatctgggaacggctgaggccggcaccttcgaaggtgtcgacttccagatcaacgacgcgaagaacggtgcccgaatcggcatccgcaactgggccgatccgaccggcgccggctatcagacggcgtcccattggggcgtgctgcgtctgctggccgattcctccgaaaccgagacccccggcggcgaggagacccctggggggggtaccgacaagcctggcgacgagaagccgcagccttccgacgatgctgacaacgacgacaagatgccgcagaccggttccgcggtcatcggagtcgccgtggtggcgttgctgctggttgccgccggatgcgggctggtcatcgctcggcgtcgatga

SEQ ID NO: 2 - DNA, 2100 bp, Bifidobacterium pseudocatenulatum
  source 1..2100: mol_type = genomic DNA
gtggcagaccttgatgcggattcgctgaacgaatcagctgaaaacacgcaggaagatcagatccagaacgatcagctcgaagatgcgcagctcgatgacaccttggctccggagcattacgacgcttccgatctgagggttctggaaggccttgaggcggtgcgaatccgcccgggcatgtacatcggctccaccggcccccgaggcttgcaccacctggtgtacgagatcgtcgacaactccgtcgatgaggcgctggcaggctacgcttcgcacatcgaagtgacgattctgccggacggcggcgtgcgcgtggtggatgacggccgaggcattccggtcgacgaagtgccgggcgaaggcgtttccggcgtggaaaccgtgatgaccaagctgcatgccggcggcaagttcggtggcggcggctatgcggtttccggcggtctgcacggcgtgggcatctccgtggtgaacgcgctgtcgacccgcgtcgacatcgaagtgcgccgacagggcctccactggacccagacctacatcgaccagaagccgaccgcacgtcttgccaagggcgagccgatgggcgaagacgagtccaccggcacttccgtgaccttctgggcagacggcgcgatcttcgaaaccaccacctacgatttcgagaccctgcgcaaccgcttccagcagatggcgttcctcaacaaggggctgaaactgtccctgaccgatttgcgcgaaccggatcaggccggagacgaagtcgcgggcgaaagcgacgacaatgccgaaccgaagcatcagacggtcacctaccaatacaacgacggcatcaaggattatgtcgattacttggtgaagtcccgcaaggcaacccccgtcgaaccggacgtgatcgatttcgaagcggaagacctgaaaatcggcatttccgcggaaatcgccatgcaatggaccaccgcatactccgaagcggtgcacaccttcgccaacaccatctccaccaccgaaggcggtacccacgaagaaggcttccgcgccgcgctgacctcgctcgtcaaccgttacgcacgtgaaaagaacatcctcaaagacaaggatgagaacctctccggcgacgacgtgcgcgaaggcctgaccgcagtggtgtcggtgaaactcaccaccccgcagttcgaaggccagaccaagaccaagctcggcaattccgaagcgaaaaccttcgtacagcgtgtgatgaccgacaagctcggcgactggttcgattcgcatcctagcgaggccaagaacatcatccagaaggccattgaagcctcccgtgcgcgtcttgcagccaagaaggcacgtgagaatacccgccgtaagtcaatcttcgaatctgcgggcatgccagacaaactgaaggattgccagtccaacaatcctgaagaatgcgaactgttcatcgtggagggcgactccgcaggcggctccgcaattcagggacgcaacccgatcacgcaggccatcctgccgttgcgaggcaaaatccttaacaccgagcgtgcaagcctcgaccgcatgatgaagtccgaaaccatcgaatcgctgatcaccgcggtcggcggcggctatggcgaggatttcgacctgaacaaagtccgctaccacaaggtcatcatcatggccgatgccgatgtggacggcgcgcatatcgcaaccctgaatctgacgctgttcttccgctacatgcgcccgatgatcaccgctggttacgtgtatgtggccatgccgccgctgtaccgactcaagtggaccaaaggcgcgcacgacttcgtgtacaccgacgccgaacgcgaccgcgtgctcgccgaaggcaagtccgccggccgtcagctgccgaagggcgaaggcatccagcgttacaagggtctgggtgaaatgagctaccaggaactgtgggaaaccaccatggatcctgaccaccgcattctgaagcaggtgcagatcgaagacgcggccgcagccgacgaaaccttctccatgctcatgggagacgaagtcgaacctcgccgtctgttcatccagcgcaacgcccgcaacgtcagctggatcgacgcgtag

SEQ ID NO: 3 - DNA, 831 bp, Bifidobacterium pseudocatenulatum
  source 1..831: mol_type = genomic DNA
atggctatccgcgtttataagccgacgactgcaggccgccgtaacgcgtccgtctcggacttctccgagcttacgcgttctacgcctgagaagtcgctggttcgcaaactcagcaagactggcggtcgtaactcttacggccgtatgacctcccgtcatcgtggcggcggtcacaagcgccagtaccgtctcatcgacttcaagcgttgggacaaggacggcgtgccggcaacggtcgctcacatcgagtacgacccgaaccgttccgcccgcatcgcactgctgcactacgcagacggtgagaagcgctacatcatcgctccggaaggtatcaagcagggtgacgtcatcgagaccggcgcccaggctgatatcaagccgggcaacaacctgccgctgcgcaacatcccgactggtaccgtggtgcacgcaatcgagctccgcccgctgggtggcgccaagatcgcccgctccgctggtgcagccgtgcagctcgtcgctaaggatggcgcttacgcccagctgcgtatgccgtccggagaaatccgcaacgtggatgctcgctgccgcgcaaccgtcggtgaggtcggcaactccgatcacgccaacatccagctcggtaaggcaggtcgtgcacgttggatgggcaagcgcccgatcacccgtggtgaatccatgaaccctgtcgatcacccgcacggcggtcgtacccgcggtggcaagccgccggtttctccgtggggcaagggcgaggttcgtacccgccgtccgaagaaggcttcgaacaagatgattgttcgtcgtcgcccgaatggtaagaaccgtaagtaa

SEQ ID NO: 4 - DNA, 1515 bp, Bifidobacterium pseudocatenulatum
  source 1..1515: mol_type = genomic DNA
ttgtcagctgaactcgaagacatccacgaggaatgcggtatttttggcgtttggggtcacccggacgccgcccgactcacctacttcggcctgcacgcgctgcagcatcgtggtcaggaaggcgccggcattgtctcgaacgataacggtcatctcatcggtcatcgcggaacgggtctgttgacccaagtgttcggcgacgaacgcgaaatcgaacgcctgaagggagacaaggcgatcggccatgtgcgttacgccactgccggttcaggcggcaccgacaacatccagccattcatcttccgcttccatgacggcgatatggccttgtgtcacaatggcaatctgacgaactgcccgactctgaggcgtcagttggaagacgaaggcgcaatcttccactccaattccgacaccgaagtgttgatgcacctgttgcgccgctccacacagcgtacgttcatggacaagctcaaggaagcgctcaacaccgtgcatggcggtttcgcctacctgatcatgaccgaagacgccatgatcggcgcgcttgatccgaacggtttccgcccgctttccctcggcaagatgaaaaacggcgcttatgtgctcgcttccgaaacctgcgcgcttgacgttgtcggcgccgaattggtgcgcaatattcgcccgggcgaaatcgtggttatcgacgatcacggctacaagatcgtgcagtacaccaatcagacccagttggccatctgctcgatggaattcatctacttcgcacgccccgattccgacatttacggcgtaaacgtgcattccgcccgcaagcgtatgggtgcgcgtctggcccaagaatcgccggtcgatgccgatatggtcattggcgtgccgaattcctcgctgtccgcggcctccggctatgcggaagaagctggtctgccaaacgagatgggcctgatcaagaaccagtatgtggctcgaaccttcatccagccgacgcaggaactgcgcgagcagggcgtgcgcatgaagctgtccgccgtgcgcggcgtggtcaaaggcaagcgcgtgatcgttatcgacgattccatcgtgcgcggtaccacgtccaagcgcatcgtgcagctgctgaaggaagctggcgccgccgaagtgcacatgcgtatcagctcgccgccgctgaagtacccgtgcttctacggcatcgacatctccaccaccaaggagctcatcgccgcaaagaagtccgttgaagaaattcgcgatttcattggcgccgattccttggcgttcctgtcactcgacggattggtcgaatctatcggcctgggtgcggacgccccgtacggcggtctgtgcgtggcctacttcaatggcgactacccgaccgcactcgacgattatgaaagtgattttttgaagtccctcaccccagaagatcgcgtgcgtctgcctgaattcgccttgtataagagcaagtacgagggcaacgaatacaccactacttcatcccaagaagaacactga

SEQ ID NO: 5 - DNA, 3561 bp, Bifidobacterium pseudocatenulatum
  source 1..3561: mol_type = genomic DNA
ttggctgaggctacgacgaacaccaccaccatcatcgcacgcgccgaccagcacgatattgatctgcacaaggcgtcggaccgtgtgaacttcggctccatccgcgagcccattgatgtaccctacctgttgggtgtacagactgacagcttcgactggctcatcggcaacgagcgctggcagaagcgtgtcgaggaggatctggcgaacggcaccaacaccgtgccccacacctccggtcttgatgaggtcttccaggagatctcaccgatcgagaacttcgctcagaccatgagcctgaccttctccgatccgtatttcgaagaaccgcgccacaccgtgcaggagtgcaaggagaaggattacacctactccgcgccgctgtatgtgaacgctgaattcgaaaacggcgacaccggcgaaatcaagtcccagaccgtgttcatgggcgatttcccgctgcagaccccgcacggcaccttcatcatcggtggtaccgagcgagtgatcgtgtctcagctggtgcgttctccgggcgtgtacttcgaccgcagccaggatcgcacttccgacaaggaagtcttcggcgcgaagatcatcccgagccgtggcgcatggcttgagttcgagatcgacaagcgtgacgtgcttggcgtgcgcgtggaccgcaagcgcaagcagtccgccatcgtgttcctcatggccatcggcatgaccaaggatgagatcgccgatgcgttcagggattacccgctggttatggacgcgcttgccaaggagaccgtgcagacccaggacgaggctctgaccgatctgtaccgcaagatccgcccggccgacaccccgacgccggaagctggccgcaacctgctggattccttctacttcaacaccaagcgttacgatctggcccgcgttggccgttacaagatcaaccgcaagcttggtctggaaaaggatgtcaacgatcgcagcctgtctcgcgaagacatcatctccaccatcaagtacctggtcaccctgcatgccggcgacaccaagttcccgggcaagcgtgacggccaggatgtggatctgcgcgtggacgtcgacgatatcgatcatttcggcaaccgtcgtatccgccaggtcggcgaactgatccagaaccagctgcgtaccggtctgagccgtatggagcgtgtggtccgcgaacgtatgaccacccaggatccggaggccatcaccccgcagtccctgatcaacattcgtccggtgaacgccaccatcaaggagttcttcggaacttcccagctgtcgcagttcatggatcagaacaacccgttggcaggcgtcaccaacaagcgtcgtctgtccgctctgggccctggcggtctgtctcgtgaccgcgcatccatggaagtgcgagacgtgcacccgtcccacttcggccgtatgtgcccgatcgaatctcctgaaggtccgaacatcggtcttatcggttctctggcaaccttcggccgcatcaatccgttcggcttcatcgagaccccgtaccgtaaggtcatcaacggccatgtgaccgacgaggtcgaatacatgaccgcagaccgcgatgccgagcacgtgatcgcacaggccaaccaggaactcgacgagaacggcaacttcgtcaagaagcaggctcttgcccgagtcggcgaagaagaagcagtcgatgtgcccgtcagctccgttgactacatggacgtttccccgcgtcagatggtttccgtcggcgcctccctgattccgttcctggagcacgatgagggccaccgagcgctgatgggtaccaacatgcagcgtcaggcagtgccgctgatcgaatccgagcgcccgctggtgggcaccggtgccgaatggcgtgcggccgtcgattccggcgatgtcattctggctgagaagccgggtgtggtgacgtatgtttccgccgacatcatccgtgtgatgaacgacgacggcaccaccagctcctacaagctggccaagttcctgcgttccaaccagaccacctgctacaaccaggttccgctgatccacgacggcgaacgtgtggaagccggtaccgtgcttgccgatggtccggccacccagaagggcgaaatggcactgggcaagaacctgctcatcgccttcatgccgtggaacggctacaactacgaggatgctgtgatcatctcccagcgtctcgtgcaggacgacaccctgagctccatccacatcgaggaatatgagatcgacgcccgcgaaaccaagctgggtgccgaagagatcacccgcgatctgccgaacgtcggcgaggacgcggtggccaacctcgacgagcgtggcatcattcgcatcggtgccgaggtcgaagccggcgacattctggtgggcaaggtcaccccgaagggcgagaccgagctgactccggaagagcgtctgctccgcgccatcttcggcgagaagagccgcgaggtgcgtgacacctcgctgcgcgtgcctcacggcgaaaccggtacggtgatcgccgtcaaggagatcactcgcgaggatgccgaggaagacggcgacgagctgccgaacggcgtgaaccagatgatccgcgtctacatcgcgcagcatcgtaagatcacccagggagacaagctgtccggccgccacggcaacaagggtgttatctcccgcattctgccggaagaggatatgccgttccttgccgacggtactccggtcgacatcatgctgaacccgctgggcgtgccttctcgaatgaaccttggccaggtgctggaactgcacttgggctggatcgcgcacgccggctgggacatctcccttgatccggatgccgaagccgcttggaagaagtacattccgcagggcgccgaaaagggcgagccgggcactccggtggcaaccccggtgttcgacggcgttcgtccggaaaccatcaagggcctgctgtcctgcacccttccggatcgcgacggcaacaagctggtcggcgacgacggcaaggctgtgctgttcgacggccgtaccggcgaaccgtatccgaagccgatctccgttggctacatgtacatgctgaagctgcaccacctagtcgacgacaagatccacgcgcgttccactggcccgtactccatgatcacccagcagccgttgggcggtaaggctcagttcggtggccagcgtttcggcgagatggaagtgtgggccctcgaggcctatggcgccgcctacacgctgcatgaaatgatgaccaccaagtccgatgacgtcgacggccgcgtgcgtgtctacggcgccatcgtgaagggcgacaacctgccgccggcaggcattccggaatccttcaaggtgctgcttaaggaaatgcagtccctgtcgctgaacgtcgaagtgctcaacgccgaaggcgtggccatcgacatgaaggacgaggacgacgatccgtctacttcctccgacgatttgggcttcaacattggcgcacgtcctgacgcggccgccaaggaagaccaggttgtggaagaacctgaattccagtga

SEQ ID NO: 6 - DNA, 2586 bp, Bifidobacterium pseudocatenulatum
  source 1..2586: mol_type = genomic DNA
atgttcgaacggtttaccgaccgtgcgcggcgcgtgatcgtgctggcgcaggaagaggctcgtaccctccagcacaactacatcggtaccgagcatctgctgcttggcctgattcgtgagggtgacggcgtcgcagccaaggcgctggcctcaaagggtgtgaccttggatgacacccgcaaacaggtcgaagagatgatcggtaaggggaatgccacgccgaacggccacattcccttcaccccgcatgccaggcaggtgttggagctgtcgctgcgtgaggcgttgcagctggggcacagctatatcggcaccgagcatatcctgctcggtctgattcatgaaggcgaaggcgtcggcacccaggtgctgatcaagatggacgtcaatcttggcgagctgcgcagcgccaccatcgacctgatccgtggcaattccggtgatggcaagggcgatggcaagggcgatttggccaatgccggtggcgtgcaggatcgtcgcaaccagaccggttccgcgattcttgaccagttcggccgcaatctgaccgctgaagctgccgccggcaagcttgatccggtgattgggcgttcgagtgagatcgagcgtgtgatggtggtgctgagccgccgtaccaagaacaatccggtgctgatcggcgagccgggtgtcggcaagacggccgtggtcgaaggcttggcgcagaagatcaatgccggcgacgttccggagacgctgaagggcaagcaggtctattcgttggatctgggatccatggtggctggttcgcggtatcgtggcgatttcgaggagcgtctgaagaaggtgctcaaggagatcaagacccgcggcgacatcgtgctgttcatcgatgagatccataccattgtgggcgctggttccgcggatggcgctcttggcgcttccgacatgttgaagccaatgctcgcgcgaggtgagctgcagaccattggcgccaccaccaccgacgagtaccgtaagtacatcgagaaggatgccgctttggaacgtcgtttccagcccatccaggtgcatgagccgagcattgccgaaaccatcgagatccttaagggcttgcgttcgcgttacgagaaccatcaccatgtgacgatcaccgatggtgcgttgcaggccgcggccgatctgtcgagccgttacattcaggaccgtcatctgccagacaaggccatcgatctgatcgatgaggccggtgcgcgtctgcgcatccgtcgtctgaccgctccgccggagcttaaggaacttgacacgaagatcgccaagcttgccgaagagaaggaccaggccatcaagggccaggacttcgaaaaggccgctgagctgcgtgataagcaggagaagctggaagccgaacgcaagcagaaggaatcttcgtggcgtgagggcgaatccgatgtgaagatggttgtggatgaggatgtcatcgccgaagtgatttcccagaccaccggcattccggtgttcaagctcacccaggccgagtccaagaagctcatgaccatggaaagcgagctgcacaagcgcatcatcggccaggacgaggccgtgtccgcgttgagccgctccatccgtcgtgctcgtgttggtttgaaggatccgaagcgtccgtccggttcgtttatcttcgctggccccaccggcgtcggtaagaccgagctggccaagacgctcgccgaattcctgtttgacgacgaggacgcactgattcgtgtcgacatgtctgaattctccgagaaatatgcggcttcgcgcctatttggtgctcctccgggatacgtcggttacgaagagggcggcgaactcaccgagaaggttcgtcgcaagccgttctccgtggtgctgttcgatgagatcgaaaaggcccatccggatatcttcaacacgctgctgcaggtgcttgatgacggtcatctgactgatggccagggccgcaaggtggacttcaagaacaccatcatcattctgaccaccaatcttggtacgcgagacatcgccaaggccgccaacaccggcttcaacttgggtgccaacaccgagtcgagctaccagcgcatgaaggatcaggtttccgcggagctgaagcagcagttccgtccggaattcctgaaccgtctggacgacatcatcgtgttcaagcagctcaccgagccgcaagtgcgtcagatcgtcgatcttgacgtcaagcagctcaatgatcgcttgttcgatcgccacatgtccctcgagcttaccgacgctgccaaggatctgctcgcgcagaagggcttcgacccgctgctgggcgcgcgtccgttgcgtcgcgtgattcagcgcgacgtcgaagacgccatttcggagaagatcctgatgggcgaactcgaagatggccagcgcgtgaaggtcgatgcggaaggcgaaggcatcctgggcgagttcacctttaccggtgaggcgttcgaagagccaaatacggagcctgctgaaggtgaagtcgcagctgaaaccgaggcacctgccgaatcgacggaatcgacagaacttacggaatccgcagaatctgttgaataa

SEQ ID NO: 7 - DNA, 2130 bp, Bifidobacterium pseudocatenulatum
  source 1..2130: mol_type = genomic DNA
atggcactagacgtgctcaatgatctcaaccagatccgtaacatcggcatcatggctcacatcgatgccggtaagaccactaccaccgaacgtatcctgtactacaccggcaagaactacaagatcggcgagacccatgacggtgcctcgacgatggacttcatggctcaggagcaggaacgcggcatcaccatccagtccgctgcaaccacttgcttctggaaccgtcagacccatgacgagaagcagaagttccagatcaacatcatcgataccccaggccacgtggacttcacggccgaggtggagcgctccctgcgcgtgctcgatggtgccgttgccgtgttcgacggcaaggaaggtgtggagccgcagtccgagaccgtgtggcgtcaggctgacaagtacggcgttccgcgtatctgcttcatcaacaagatggataagctcggcgctgacttctactactccgtcgacaccatcaaaaccaagctgggcgcgaccccgcttgtcgtgcagctgccgatcggcgctgagaacgacttcgctggcgttgtcgatctgattcgtatgaaggcttacgtctggaacgacgtttccggcgacatgggcgctcactacgacactaccgacatccccgccgacctgcaggacaaggccgagcagtatcgtgcagagctgctcgaccaggtcgcagaatccgacgaagagctgcttgagaagtatctcgagtccggcgaactgactgaggacgagatccgtagcggcatccgtaagctcaccattaaccgtgaagcctacccggtgctctgcggctccgccttcaaggacaagggtgttcagccgatgctggacgccgtcgtcgactacctgccgagcccggaggacgttccgtccatcgtcggtttcgatcctaaggacgaatccatcgagatcgatcgcaagccgaccaccgatgatccgttctctgccctggtcttcaagatctctacccacccgttctacggcaagctcgtgttcgtgcgcgtctactccggcgccgtcaccccgggcgacaccgtgcttgactccaccaagggcaagaaggaacgcgtcggcaagatcttccagatgcacgccgacaaggagaacccggtcgatgccgccgaagccggcaacatctacaccttcgtgggcctgaagaacatcaccaccggtgacaccctgtgcgacgaaaaggcgcctatctccctcgaatccatgaccttcccggatccggtgatcgaggtggccgtggagccgaagaccaaggccgatcaggagaagatgagcatcgctctggcgaagctgtccgacgaagatccgaccttccaggtgaagaccgacgaagagtccggccagaccctgatctccggcatgggcgagctgcagctcgacatcatcgtcgaccgtatgcgtcgtgaattcaaggtggagtgcaacgtgggtaacccgcaggttgcataccgtgagacgatccgcaaggccgtcatgaaccaggaatacacgcacaagaagcagaccggtggttccggccagttcgcaaaggtcttgatgaacttcgagccgctcaacaccgaagagggcgagacctacgagttcgtcaacgaggtcaccggtggccacatcaccaaggaattcattccttccatcgatgctggtgtgcaggaagccatggaatccggcgtgctcgccggcttcccggtggttggcgtcaaggctaccgtcactgacggccaggtccacgacgtcgattcctccgaaatggccttcaagatcgcaggttccatgtgcttcaaggaagctgctccgaaggccaagccggtcatcctcgagccgatcatggccgtggaagtgcgtactccggaagagtacatgggcgacgtgatgggcgatatcaacgcccgtcgtggttccatccagtccatgaccgactccaccggtgtcaaggtcatcgatgccaaggttccgctgtccgaaatgttcggctacatcggcgaccttcgctccaagacccagggccgcgcaatgttcaccatgcagatggactcctacgctgaggttccgaagaacgtctccgaggagatcatcaaggcccagcgcggcgagtga

SEQ ID NO: 8 - DNA, 3312 bp, Bifidobacterium pseudocatenulatum
  source 1..3312: mol_type = genomic DNA
gtgagcgaaaacaacgtgtatccgaaggcagctgcgggtgagcagagcgccaatgtagcgccgaaccccagtttcccgaagctggaagaatccgtccttgattattgggagaaggacgacactttccagaagtccattgaacgccgtccttccggcgatcacagccagaacgaattcgtcttcttcgacggaccgccgttcgccaacggcctgccgcactacggccacctgctgaccggctacgccaaggatgtgattccgcgctaccagaccatgaagggccacaaggtcaatcgtgtgttcggctgggatacgcacggtctgccggccgagcttgaagcccagaaggaactgggcatcgactcggtcgatcaggtcaaggaaatgggcatcgacaagttcaacgacgcttgccgcgcctccgtgctcaagtacaccaacgagtggaaggactacgtgcaccgtcaggcacgttgggtcgatttcgagcatggctacaagacgctgaacattccatacatggaatccgtgatgtgggcgttcaagcagctgtacgacaagggcctcgcatatcagggctaccgcgtgctgccgtactgtccgaaggatcagacgccgctttccgcgcacgagctgcgcatggacgccgacgtgtatcaggatcgtcaggacaccaccgtgtccgtggccgtgaagctgcgcgacgaggaagacgcctatgcggtgttctggaccaccacgccgtggaccgttcccaccaacttcgccatcgtggtcggcgcagacatcgactatgtggaagtgcgtccgaccgaaggcaagttcgcgggcaagaagttctacctgggcaagccactgctcggctcctacgccaaggaacttggcgacaactatgagatcgtgcgcgaactcaagggtgccgagatggaaggctggcgctactacccggtgttcccgtacttcgcaggcgacgagaacgccgtcgaaggcaaggttccgggtccggaaggctatcagatcttcaccgccgactatgtcgataccgttgagggtaccggtctcgtgcaccaggctccgtacggcgaggacgatatgaacacgctcaacgccaagggcatcaagagcgttgacgtgctcgacgcgggctgcaagttcaccgcgctgtgcccggactacgagggcatgtacgtgttcgatgcgaacaagccgattctgcgtaacctgcgtgccggtgacggtcctctggagcgtattccggaagatcagcgcgcgatccttttccaggagaagagctacgtgcactcctacccgcactgctggcgttgcgccacgccgctcatctacaagccggtgagctcgtggttcgtgtccgtcaccaagatcaaggatcgtctgctcgaactgaaccaggaaatcaactggattccgggcaatgtgaaggacggccagttcggcaagtggctggccaacgcccgtgactggtcgatctcccgcaaccgtttctggggttcgccgattccggtgtgggtttccgatgatccgaagtatccacgcgttgacgtgtacggttcgttggacgagctgaaggctgattttggcgattatccgcgcgaccatgagggcaatgtcaacatgcaccgcccgtacatcgacgagctgacccgcgtcaacccggacgatccgaccggcaagagccacatgcaccgcatcaccgacgtgatggactgctggttcgaatccggttccatgagcttcgcccagtaccattacccgttcgaaaacaaggaaacgttcgaacagcatttcccgtgcgattacatcgtggaatacatcggccagacccgtggctggttctacgtgcagcacatcatggcgaccgcactgttcgacaagccggcgttcaagaacgtgatctgccatggcatcgtgcttggctccgacggccagaagatgtcgaagcatctgcgcaactacccggatgtgaatggagtgttcaacgatttcggctccgacgccatgcgctggttcctcatgagctcgccgatcctgcgcggcggcaacctgatcgtgaccgccgatggcattcgcgacaccgtgcgtcaggtcatgctgccagtgtggagttcgtactacttcttcaccctgtatgcgaacgccgccaataatggcgccggcttcgatgctcgtacattgcgtgccgatgaggtcgccgcactgccggaaatggatcgttacctgctggcgcgtacccgccgactgatcgagaagacgcaaagctcgctggacaacttcctgatctctgacgcatgcgaagccgtgtccgatttcattgacatgctcaccaactggtatatccgcaacaatcgtgaccgtttctggaatgaggatgcgaacgcgttcaacacgctgtacaccgtgcttgaagcattcatgcgcgtgatcgcaccgcttgctccgatggaagcggaagcagtgtggcgtggtctgaccggtggcgaatccgtgcacttggccgactggccgttccttgccgacgagcagaccggagaggcaacagaactgggccgcgtgcttgttgacgatccggctctggttgatgcgatggagaaggtgcgcgaggtcgtgtccggcactctgtctatgcgtaagacaaagcagatccgtgtgcgccagccgctgtccaagctgaccgtggtggtggagaacactgccgccgtggccgcatacgacgagattctgaaatccgaactgaacgtgaagaacgttgaattgtgcacgcttgaagatgccgaagcccaaggcttgaagatcatcaacgagctgcgtgtgaacgctcgcgtggcaggcaagcgcctgcgcaaggacgtgcagttcgccatcaaggcttccaagtccggcgcatggcatgtgaacgccgaaggcgctccggtatgtgagactccgaacggtgagatcgtgcttgaggaaggcgaatatgagctgatcaacagcgtggaggagaagaacgccgaagaggccgccaactctgtaagtgctgcactgccgaccggtggcttcgtgatcctcgacaccgagctgaacgacgatctgatcgcagaaggctatgcccgcgacgtgatccgcgccgtgcaggacgcccgcaaggccgccgatctgcagatctccgaccgtatcgcactgaagctcgttgtgcccgccgaagacgtggccaaggtcgaacagttcaaggaacttgtctcctccgagacgctcgccacttccttcgaagtgactgccggcgatgagctgaacgttgaggttgccaaggcctga

SEQ ID NO: 9 - DNA, 2091 bp, Bifidobacterium pseudocatenulatum
  source 1..2091: mol_type = genomic DNA
atggctgactcactcgcatcgcagatcatcactgcaatcggtggtcctgaaaacgttcgcagtctgacgcattgcgccactcgactgcgctttgaactggttgacgcatccaaggtcgatcagaatagtctcgagcacatgcagggcgtgctcggcgcggtgccgcagagcggcgaccgcttccaggtggtcatcggcggtggcgttgccaccgtgtacgaaaacatcatgcatctgcccgaaatggccggtgtcggcggtgcctccgcatccgacgatggtcagaagagcaatgccgacgtcaaggccgaagcccgttccaaggcccgcggcaaggtggcttggctggactccttcttcgagtatctctccgattccttccgcccgattctgggcgtgctgctcggcgcttccatcatcatcgcgctggtcaacctgcttatttcgctgaacgtcattccgaatgacgaggtttccgcaggctgggtattcgtgaaagccatctggaagggcgtattctacttcctgccgatcatggtcgcctacaacgcgtccaagaagctcaaagtcgacccatggctgggtggtgccatcatggccatgctcatgaccccgcagttcaccggcttgatggacgccaagaccaccacgtgcgtggagaacgccgctctgggcaccaagtcttgcatggccaacatattcggtctgccgatggcattgagcgactattccggcaacgtgttcgtgccgctgctcatggccgccgtgcttgctctcgtctaccacggattgaagaggatcatcccggaaagcgtccagctggtcttcgtgccgttcttctgcatgatcatcgttggcgcgctgaccgccttcatcatcggcccgatcggcgtgtgggtcggcaacggcctcggcgtcggcttggcctggatgaacacccatgccccgttcatcttcgccatcatcattccgatgctgtacccgttcctcgtgccgctcggtttgcactggccgctcaacgccctgatgctcatgaacatccagactctcggctacgacttcatccaaggcccgatgggcgtgtggaacttcgcctgcttcggcgctaccgctggcgtgctcttccttgctgtgcgtgacaaggataaggacatgcgccagaccgctttgggcgcacttgcggccggcctgctcggtggcgtttccgaaccgtctctgtacggcattcacctgcgttacaagctcatctacaagcgcatgctggtgggctgcggtctcggtggcgtcgtcatcgccatcctcggttggctcttcccgtccgtcaccgccgccggccagaccgtgcatggcgtgaccaccaccgctttcgcattcacctcgttgctgaccattccggtcttcaatcagatgtgggtgtatgcagtgtccatcgccgtgtccttcctcacctccttccttctgatcatcaccttcgactaccgcactccggaacagaaggccgaagtgctggcccgtgcggctgccaatcagaagaccgctgtctcgtcggtcgaagccaagggagtcgctccggctgctgccaccgcgactgccactgttgccgccaccaagactgaagccccggctgctgctgccaccaccaccgtggtgaacgctccagtcgcaggccatgtgatttccctggatgaaaccggcgatccggtgttcgcatcccgcgcactaggcgaaggcgtcggcatccagccggcagacagcaccgtcgtcgcgccggtatccggcgtgctgcagaccgtcgccgaaaccggtcacgcattcggcatcaaaaccgatgatggcgcggaagtgctcgtgcacgtcggcatcgacacggtgaagatgaacggcgaaggcttcgatgtgaaggtcaaggccaacgaacacgtgaacgcgggggacaacctcgttgtcgtcgactttgataaggttaaggaagctggatacagcaccaccacattgatgacggtgctgaacacagtggccttcgcgtccgtcacgccaaagaccggcgtcgacgtcaaggccggtgagtcggtgatcgacattcagcgctga

SEQ ID NO: 10 - DNA, 21 bp, synthetic construct
  source 1..21: mol_type = other DNA
gggcaagatcggcatcatcta

SEQ ID NO: 11 - DNA, 21 bp, synthetic construct
  source 1..21: mol_type = other DNA
cacattggtggtgttcacgtc

SEQ ID NO: 12 - DNA, 22 bp, synthetic construct
  source 1..22: mol_type = other DNA
cgagaatgcgaacacgtacttc

SEQ ID NO: 13 - DNA, 22 bp, synthetic construct
  source 1..22: mol_type = other DNA
ctgctcggtgttgtaatcgttg

SEQ ID NO: 14 - DNA, 28 bp, synthetic construct
  source 1..28: mol_type = other DNA
tcctgtggatttcgacggtgacgagcag

SEQ ID NO: 15 - DNA, 28 bp, synthetic construct
  source 1..28: mol_type = other DNA
gagtgcggttgatggtgcatacggcaag